European Patent Application EP 4 410 987 A1, published August 7, 2024. Title: An AAV9 capsid variant for targeted gene transfer. Applicant: Universitätsklinikum Hamburg-Eppendorf. The sequence listing filed with the application follows.

SEQUENCE LISTING (29 sequences)

SEQ ID NO: 1 - protein, 6 aa, synthetic construct
GGNYXX

SEQ ID NO: 2 - protein, 7 aa, synthetic construct
GGNYGLG

SEQ ID NO: 3 - protein, 7 aa, synthetic construct
GGNYGWG

SEQ ID NO: 4 - protein, 7 aa, synthetic construct
GGNYGVG

SEQ ID NO: 5 - protein, 7 aa, synthetic construct
GGNYGFG

SEQ ID NO: 6 - protein, 7 aa, synthetic construct
GGNYGSG

SEQ ID NO: 7 - protein, 7 aa, synthetic construct
GGNYGCG

SEQ ID NO: 8 - protein, 7 aa, synthetic construct
GGNYGGG

SEQ ID NO: 9 - protein, 7 aa, synthetic construct
GGNYGAG

SEQ ID NO: 10 - protein, 7 aa, synthetic construct
GGNYGYG

SEQ ID NO: 11 - protein, 7 aa, synthetic construct
GGNYGWV

SEQ ID NO: 12 - protein, 7 aa, synthetic construct
GGNYGLV

SEQ ID NO: 13 - protein, 7 aa, synthetic construct
GGNYGLC

SEQ ID NO: 14 - protein, 7 aa, synthetic construct
GGNYGLF

SEQ ID NO: 15 - protein, 7 aa, synthetic construct
GGNYGMC

SEQ ID NO: 16 - protein, 7 aa, synthetic construct
GGNYGLI

SEQ ID NO: 17 - protein, 7 aa, synthetic construct
GGNYGGL

SEQ ID NO: 18 - protein, 7 aa, synthetic construct
GGNYGVD

SEQ ID NO: 19 - protein, 7 aa, synthetic construct
GGNYGFV

SEQ ID NO: 20 - protein, 7 aa, synthetic construct
GGNYDFG

SEQ ID NO: 21 - protein, 7 aa, synthetic construct
GGNYALG

SEQ ID NO: 22 - protein, 7 aa, synthetic construct
GGNYVLG

SEQ ID NO: 23 - protein, 7 aa, synthetic construct
GGNYCLA

SEQ ID NO: 24 - protein, 7 aa, synthetic construct
GGNYGXX

SEQ ID NO: 25 - protein, 7 aa, synthetic construct
GGNYXXG

SEQ ID NO: 26 - protein, 7 aa, synthetic construct
GGNYXXX

SEQ ID NO: 27 - protein, 7 aa, synthetic construct
GGNYGXG

SEQ ID NO: 28 - DNA, 19 bp, synthetic construct
  source 1..19: mol_type = other DNA
gggactttcctacttggca

SEQ ID NO: 29 - DNA, 19 bp, synthetic construct
  source 1..19: mol_type = other DNA
ggcggagttgttacgacat